European Patent Specification EP 3 765 056 B1, published August 2, 2023. Title: COMPOSITIONS, METHODS AND USES OF TENEURIN C-TERMINAL ASSOCIATED PEPTIDE-1 (TCAP-1) FOR TREATING OPIOID ADDICTION. Applicant: SLEE, Andrew STEIN, Robert ARMEN, Garo. Application Not yet assigned. The sequence listing filed with the application follows.

SEQUENCE LISTING (12 sequences)

SEQ ID NO: 1 - protein, 41 aa, Artificial Sequence
  Mouse TCAP1 (41 a.a.)
QQLLGTGRVQGYDGYFVLSVEQYLELSDSANNIHFMRQSEI

SEQ ID NO: 2 - protein, 41 aa, Artificial Sequence
  Human TCAP1 (41 a.a.)
QQLLSTGRVQGYDGYFVLSVEQYLELSDSANNIHFMRQSEI

SEQ ID NO: 3 - protein, 41 aa, Artificial Sequence
  G. gallus TCAP-1
QQLLNTGRVQGYDGYFVLSVEQYLELSDSANNIHFMRQSEI

SEQ ID NO: 4 - protein, 40 aa, Artificial Sequence
  Mouse TCAP1 (40 a.a.)
QLLGTGRVQGYDGYFVLSVEQYLELSDSANNIHFMRQSEI

SEQ ID NO: 5 - protein, 43 aa, Artificial Sequence
  Mouse preTCAP1 (43 a.a.)
QLLGTGRVQGYDGYFVLSVEQYLELSDSANNIHFMRQSEIGRR

SEQ ID NO: 6 - protein, 44 aa, Artificial Sequence
  Mouse preTCAP1 (44 a.a.)
QQLLGTGRVQGYDGYFVLSVEQYLELSDSANNIHFMRQSEIGRR

SEQ ID NO: 7 - protein, 40 aa, Artificial Sequence
  Human TCAP1 (40 a.a.)
QLLSTGRVQGYDGYFVLSVEQYLELSDSANNIHFMRQSEI

SEQ ID NO: 8 - protein, 43 aa, Artificial Sequence
  Human preTCAP1 (43 a.a.)
QLLSTGRVQGYDGYFVLSVEQYLELSDSANNIHFMRQSEIGRR

SEQ ID NO: 9 - protein, 44 aa, Artificial Sequence
  Human preTCAP1 (44 a.a.)
QQLLSTGRVQGYDGYFVLSVEQYLELSDSANNIHFMRQSEIGRR

SEQ ID NO: 10 - protein, 41 aa, Artificial Sequence; identical to SEQ ID NO: 1
  Mouse TCAP1 (41 a.a.)
  MOD_RES (1)..(1): optionally pyroglutamic acid
  MOD_RES (41)..(41): optionally amidated

SEQ ID NO: 11 - protein, 41 aa, Artificial Sequence; identical to SEQ ID NO: 2
  Human TCAP1 (41 a.a.)
  MOD_RES (1)..(1): optionally pyroglutamic acid
  MOD_RES (41)..(41): optionally amidated

SEQ ID NO: 12 - protein, 41 aa, Artificial Sequence; identical to SEQ ID NO: 3
  G. gallus TCAP-1
  MOD_RES (1)..(1): optionally pyroglutamic acid
  MOD_RES (41)..(41): optionally amidated